European Patent Application EP 4 450 633 A2, published October 23, 2024. Title: NON R-GENE MEDIATED RESISTANCE. Applicant: Rijk Zwaan Zaadteelt en Zaadhandel B.V. Application EP EPPCT/EP2016/000791, filed May 16, 2016. The sequence listing filed with the application follows.

SEQUENCE LISTING (8 sequences)

SEQ ID NO: 1 - DNA, 58 bp, Spinacia oleracea
  misc_feature 1..58: note = source = /organism="Spinacia oleracea" /mol_type="unassigned DNA"
  source 1..58: mol_type = genomic DNA
cctaatggctctaaggtttcatcaagacctaagaaagcagaaaaaatgcagaagccca

SEQ ID NO: 2 - DNA, 58 bp, Spinacia oleracea
  misc_feature 1..58: note = source = /organism="Spinacia oleracea" /mol_type="unassigned DNA"
  source 1..58: mol_type = genomic DNA
cctaatggctctaaggtttcatcaaaacctaagaaagcagaaaaaatgcagaagccca

SEQ ID NO: 3 - DNA, 80 bp, Spinacia oleracea
  misc_feature 1..80: note = source = /organism="Spinacia oleracea" /mol_type="unassigned DNA"
  source 1..80: mol_type = genomic DNA
attgtacaaatttcagaaacagttataaccaatttcagataataaacagatttccacttcacatatttcttacctcaarc

SEQ ID NO: 4 - DNA, 80 bp, Spinacia oleracea
  misc_feature 1..80: note = source = /organism="Spinacia oleracea" /mol_type="unassigned DNA"
  source 1..80: mol_type = genomic DNA
attgtacaaatttcagaaacagttataaccaaattcagataataaacagatttccacttcacatatttcttacctcaarc

SEQ ID NO: 5 - DNA, 83 bp, Spinacia oleracea
  misc_feature 1..83: note = source = /organism="Spinacia oleracea" /mol_type="unassigned DNA"
  source 1..83: mol_type = genomic DNA
cataaacattccgtatgagtagtactctatttgtctcaaaaagaaaattgaaaattgccctagtcgaaattttatctgcacta

SEQ ID NO: 6 - DNA, 82 bp, Spinacia oleracea
  misc_feature 1..82: note = source = /organism="Spinacia oleracea" /mol_type="unassigned DNA"
  source 1..82: mol_type = genomic DNA
cataaacattccgtatgagtagtactctatttgtctcaaaaagaaaattgaaaattgcctagtcgaaattttatctgcacta

SEQ ID NO: 7 - DNA, 49 bp, Spinacia oleracea
  misc_feature 1..49: note = source = /organism="Spinacia oleracea" /mol_type="unassigned DNA"
  source 1..49: mol_type = genomic DNA
gatgctcagccgctcaccagtatttggttttcatgagccaaaaactgga

SEQ ID NO: 8 - DNA, 49 bp, Spinacia oleracea
  misc_feature 1..49: note = source = /organism="Spinacia oleracea" /mol_type="unassigned DNA"
  source 1..49: mol_type = genomic DNA
gatgctcagccgctcaccagtatctggttttcatgagccaaaaactgga